European Patent Application EP 4 744 728 A2, published May 20, 2026. Title: Anti-Dengue Virus Antibodies, Polypeptides Containing Variant Fc Regions, And Methods Of Use. Applicant: Chugai Seiyaku Kabushiki Kaisha. Application EP, filed September 15, 2017. The sequence listing filed with the application follows.

SEQUENCE LISTING (109 sequences)

SEQ ID NO: 1 - protein, 132 aa, Homo sapiens
QVQLVQSGPDVEKPGASVKVSCKASGYTFTSNYIHWVRQAPGQGLEWMGVINPRGGSTASAQKFQGRITMTRDTSTSTVYMELSSLRSDDTAVYYCARGGRALFYDSYTTPRDGGSWWFDPWGQGSLVTVSS

SEQ ID NO: 2 - protein, 132 aa, synthetic construct
  source 1..132: note = VH
QVQLVQSGPDVEKPGASVKVSCKASGYTFTSNYIHWVRQAPGQGLEWMGVINPRGGSRASAQKFQGRITMTRDTSTSTVYMELSSLRSEDTAVYYCARGGRALFYDSYTTPFDGGSWWFDPWGQGSLVTVSS

SEQ ID NO: 3 - protein, 132 aa, synthetic construct
  source 1..132: note = VH
QVQLVQSGPDVEKPGASVKVSCKASGYTFTSNYIHWVRQAPGQGLEWMGVINPRGGSRRSAQKFQGRITMTRDTSTSTVYMELSSLRSEDTAVYYCARGGRALFYDSYTTPFDGGSWWFDPWGQGSLVTVSS

SEQ ID NO: 4 - protein, 132 aa, synthetic construct
  source 1..132: note = VH
QVQLVQSGPDVEKPGASVKVSCKASGYTFTSNYIHWVRQAPGQGLEWMGVINPRGGSRRSAQKFQGRITMTRDTSTSTVYMELSSLRSEDTAVYYCARGGRALFYDSYTTPRDDGSWWFDPWGQGSLVTVSS

SEQ ID NO: 5 - protein, 132 aa, synthetic construct
  source 1..132: note = VH
QVQLVQSGPDVEKPGASVKVSCKASGYTFTSNYIHWVRQAPGQGLEWMGVINPRGGSRRSAQKFQGRITMTRDTSTSTVYMELSSLRSEDTAVYYCARGGRALFYDSYTTPRDLGSWWFDPWGQGSLVTVSS

SEQ ID NO: 6 - protein, 132 aa, synthetic construct
  source 1..132: note = VH
QVQLVQSGPDVEKPGASVKVSCKASGYTFTSYYMHWVRQAPGQGLEWMGVINPRGGSRRSAQKFQGRITMTRDTSTSTVYMELSSLRSEDTAVYYCARGGEALFYDSYTTPFDGGSWWFDPWGQGSLVTVSS

SEQ ID NO: 7 - protein, 107 aa, Homo sapiens
DIQLTQSPSSLSASVGDRVTFTCQASQDIRKYLNWYQQKPGKAPKLLIYDASNLKTGVPSRFSGSGSGTDFTFTISSLQPEDVATYYCQQFDDLPITFGQGTRLQIK

SEQ ID NO: 8 - protein, 107 aa, synthetic construct
  source 1..107: note = VL
DIQLTQSPSSLSASVGDRVTFTCQASQDIRKYLNWYQQKPGKAPKLLIYDASNLKFGVPSRFSGSGSGTDFTFTISSLQPEDVATYYCQQFDALPITFGQGTRLQIK

SEQ ID NO: 9 - protein, 107 aa, synthetic construct
  source 1..107: note = VL
DIQLTQSPSSLSASVGDRVTFTCQASQDIRQYLNWYQQKPGKAPKLLIYDASNLKFGVPSRFSGSGSGTDFTFTISSLQPEDVATYYCQQFSALPITFGQGTRLQIK

SEQ ID NO: 10 - protein, 107 aa, synthetic construct
  source 1..107: note = VL
DIQLTQSPSSLSASVGDRVTFTCQASQEIRKYLNWYQQKPGKAPKLLIYDASELKTGVPSRFSGSGSGTDFTFTISSLQPEDVATYYCQQFEDLPITFGQGTRLQIK

SEQ ID NO: 11 - protein, 5 aa, Homo sapiens
SNYIH

SEQ ID NO: 12 - protein, 5 aa, synthetic construct
  source 1..5: note = HVR-H1
SYYMH

SEQ ID NO: 13 - protein, 17 aa, Homo sapiens
VINPRGGSTASAQKFQG

SEQ ID NO: 14 - protein, 17 aa, synthetic construct
  source 1..17: note = HVR-H2
VINPRGGSRASAQKFQG

SEQ ID NO: 15 - protein, 17 aa, synthetic construct
  source 1..17: note = HVR-H2
VINPRGGSRRSAQKFQG

SEQ ID NO: 16 - protein, 23 aa, Homo sapiens
GGRALFYDSYTTPRDGGSWWFDP

SEQ ID NO: 17 - protein, 23 aa, synthetic construct
  source 1..23: note = HVR-H3
GGRALFYDSYTTPFDGGSWWFDP

SEQ ID NO: 18 - protein, 23 aa, synthetic construct
  source 1..23: note = HVR-H3
GGRALFYDSYTTPRDDGSWWFDP

SEQ ID NO: 19 - protein, 23 aa, synthetic construct
  source 1..23: note = HVR-H3
GGRALFYDSYTTPRDLGSWWFDP

SEQ ID NO: 20 - protein, 23 aa, synthetic construct
  source 1..23: note = HVR-H3
GGEALFYDSYTTPFDGGSWWFDP

SEQ ID NO: 21 - protein, 11 aa, Homo sapiens
QASQDIRKYLN

SEQ ID NO: 22 - protein, 11 aa, synthetic construct
  source 1..11: note = HVR-L1
QASQDIRQYLN

SEQ ID NO: 23 - protein, 11 aa, synthetic construct
  source 1..11: note = HVR-L1
QASQEIRKYLN

SEQ ID NO: 24 - protein, 7 aa, Homo sapiens
DASNLKT

SEQ ID NO: 25 - protein, 7 aa, synthetic construct
  source 1..7: note = HVR-L2
DASNLKF

SEQ ID NO: 26 - protein, 7 aa, synthetic construct
  source 1..7: note = HVR-L2
DASELKT

SEQ ID NO: 27 - protein, 9 aa, Homo sapiens
QQFDDLPIT

SEQ ID NO: 28 - protein, 9 aa, synthetic construct
  source 1..9: note = HVR-L3
QQFDALPIT

SEQ ID NO: 29 - protein, 9 aa, synthetic construct
  source 1..9: note = HVR-L3
QQFSALPIT

SEQ ID NO: 30 - protein, 9 aa, synthetic construct
  source 1..9: note = HVR-L3
QQFEDLPIT

SEQ ID NO: 31 - protein, 30 aa, Homo sapiens
QVQLVQSGPDVEKPGASVKVSCKASGYTFT

SEQ ID NO: 32 - protein, 14 aa, Homo sapiens
WVRQAPGQGLEWMG

SEQ ID NO: 33 - protein, 32 aa, Homo sapiens
RITMTRDTSTSTVYMELSSLRSDDTAVYYCAR

SEQ ID NO: 34 - protein, 32 aa, synthetic construct
  source 1..32: note = FR-H3
RITMTRDTSTSTVYMELSSLRSEDTAVYYCAR

SEQ ID NO: 35 - protein, 11 aa, Homo sapiens
WGQGSLVTVSS

SEQ ID NO: 36 - protein, 23 aa, Homo sapiens
DIQLTQSPSSLSASVGDRVTFTC

SEQ ID NO: 37 - protein, 15 aa, Homo sapiens
WYQQKPGKAPKLLIY

SEQ ID NO: 38 - protein, 32 aa, Homo sapiens
GVPSRFSGSGSGTDFTFTISSLQPEDVATYYC

SEQ ID NO: 39 - protein, 10 aa, Homo sapiens
FGQGTRLQIK

SEQ ID NO: 40 - skipped

SEQ ID NO: 41 - protein, 17 aa, synthetic construct
  SITE 9: note = X = T or R
  SITE 10: note = X = A or R
  source 1..17: note = HVR-H2
VINPRGGSXXSAQKFQG

SEQ ID NO: 42 - protein, 23 aa, synthetic construct
  SITE 3: note = X = R or E
  SITE 14: note = X = R or F
  SITE 16: note = X = G, D or L
  source 1..23: note = HVR-H3
GGXALFYDSYTTPXDXGSWWFDP

SEQ ID NO: 43 - protein, 11 aa, synthetic construct
  SITE 5: note = X = D or E
  SITE 8: note = X = K or Q
  source 1..11: note = HVR-L1
QASQXIRXYLN

SEQ ID NO: 44 - protein, 7 aa, synthetic construct
  SITE 4: note = X = N or E
  SITE 7: note = X = T or F
  source 1..7: note = HVR-L2
DASXLKX

SEQ ID NO: 45 - protein, 9 aa, synthetic construct
  SITE 4: note = X = D, S or E
  SITE 5: note = X = D or A
  source 1..9: note = HVR-L3
QQFXXLPIT

SEQ ID NO: 46 - protein, 328 aa, synthetic construct
  source 1..328: note = CH
ASTKGPSVFPLAPSSKSTSGGTAALGCLVKDYFPEPVTVSWNSGALTSGVHTFPAVLQSSGLYSLSSVVTVPSSSLGTQTYICNVNHKPSNTKVDKRVEPKSCDKTHTCPPCPAPELLGGPSVFLFPPKPKDTLMISRTPEVTCVVVDVSHEDPEVKFNWYVDGVEVHNAKTKPREEQYNSTYRVVSVLTVLHQDWLNGKEYKCKVSNKALPAPIEKTISKAKGQPREPQVYTLPPSREEMTKNQVSLTCLVKGFYPSDIAVEWESNGQPENNYKTTPPVLDSDGSFFLYSKLTVDKSRWQQGNVFSCSVMHEALHNHYTQKSLSLSP

SEQ ID NO: 47 - protein, 328 aa, synthetic construct
  source 1..328: note = CH
ASTKGPSVFPLAPSSKSTSGGTAALGCLVKDYFPEPVTVSWNSGALTSGVHTFPAVLQSSGLYSLSSVVTVPSSSLGTQTYICNVNHKPSNTKVDKRVEPKSCDKTHTCPPCPAPEAAGGPSVFLFPPKPKDTLMISRTPEVTCVVVDVSHEDPEVKFNWYVDGVEVHNAKTKPREEQYNSTYRVVSVLTVLHQDWLNGKEYKCKVSNKALPAPIEKTISKAKGQPREPQVYTLPPSREEMTKNQVSLTCLVKGFYPSDIAVEWESNGQPENNYKTTPPVLDSDGSFFLYSKLTVDKSRWQQGNVFSCSVMHEALHNHYTQKSLSLSP

SEQ ID NO: 48 - protein, 328 aa, synthetic construct
  source 1..328: note = CH
ASTKGPSVFPLAPSSKSTSGGTAALGCLVKDYFPEPVTVSWNSGALTSGVHTFPAVLQSSGLYSLSSVVTVPSSSLGTQTYICNVNHKPSNTKVDKRVEPKSCDKTHTCPPCPAPELLGGPSVFLFPPKPKDTLMISRTPEVTCVVVDVSHEDPEVKFNWYVDGVEVHNAKTKPREEQYNSTYRVVSVLTVLHQDWLNGKEYKCKVSNWALPAPISKTISKAKGQPREPQVYTLPPSREEMTKNQVSLTCLVKGFYPSDIAVEWESNGQPENNYKTTPPVLDSDGSFFLYSKLTVDKSRWQQGNVFSCSVMHEALHNHYTQKSLSLSP

SEQ ID NO: 49 - protein, 328 aa, synthetic construct
  source 1..328: note = CH
ASTKGPSVFPLAPSSKSTSGGTAALGCLVKDYFPEPVTVSWNSGALTSGVHTFPAVLQSSGLYSLSSVVTVPSSSLGTQTYICNVNHKPSNTKVDKRVEPKSCDKTHTCPPCPAPELLAGPSVFLFPPKPKDTLMISRTPEVTCVVVDVEFEDPEVKFNWYVDGVEVHNAKTKPREEQYNSTYRVVSVLTVLHQDWLNGKEYKCKVTNKALPAPEEKTISKAKGQPREPQVYTLPPSREEMTKNQVSLTCLVKGFYPSDIAVEWESNGQPENNYKTTPPVLDSDGSFFLYSKLTVDKSRWQQGNVFSCSVMHEALHNHYTQKSLSLSP

SEQ ID NO: 50 - protein, 328 aa, synthetic construct
  source 1..328: note = CH
ASTKGPSVFPLAPSSKSTSGGTAALGCLVKDYFPEPVTVSWNSGALTSGVHTFPAVLQSSGLYSLSSVVTVPSSSLGTQTYICNVNHKPSNTKVDKRVEPKSCDKTHTCPPCPAPELLGGPSVFLFPPKPKDTLMISRTPEVTCVVVDVEFEDPEVKFNWYVDGVEVHNAKTKPREEQYNSTYRVVSVLTVLHQDWLNGKEYKCKVTNKALPAPIEKTISKAKGQPREPQVYTLPPSREEMTKNQVSLTCLVKGFYPSDIAVEWESNGQPENNYKTTPPVLDSDGSFFLYSKLTVDKSRWQQGNVFSCSVMHEALHNHYTQKSLSLSP

SEQ ID NO: 51 - protein, 328 aa, synthetic construct
  source 1..328: note = CH
ASTKGPSVFPLAPSSKSTSGGTAALGCLVKDYFPEPVTVSWNSGALTSGVHTFPAVLQSSGLYSLSSVVTVPSSSLGTQTYICNVNHKPSNTKVDKRVEPKSCDKTHTCPPCPAPEAAGGPSVFLFPPKPKDTLMISRTPEVTCVVVDVSHEDPEVKFNWYVDGVEVHNAKTKPREEQYNSTYRVVSVLTVLHQDWLNGKEYKCKVSNWALPAPISKTISKAKGQPREPQVYTLPPSREEMTKNQVSLTCLVKGFYPSDIAVEWESNGQPENNYKTTPPVLDSDGSFFLYSKLTVDKSRWQQGNVFSCSVMHEALHNHYTQKSLSLSP

SEQ ID NO: 52 - protein, 328 aa, synthetic construct
  source 1..328: note = CH
ASTKGPSVFPLAPSSKSTSGGTAALGCLVKDYFPEPVTVSWNSGALTSGVHTFPAVLQSSGLYSLSSVVTVPSSSLGTQTYICNVNHKPSNTKVDKRVEPKSCDKTHTCPPCPAPEAAAGPSVFLFPPKPKDTLMISRTPEVTCVVVDVEFEDPEVKFNWYVDGVEVHNAKTKPREEQYNSTYRVVSVLTVLHQDWLNGKEYKCKVTNKALPAPEEKTISKAKGQPREPQVYTLPPSREEMTKNQVSLTCLVKGFYPSDIAVEWESNGQPENNYKTTPPVLDSDGSFFLYSKLTVDKSRWQQGNVFSCSVMHEALHNHYTQKSLSLSP

SEQ ID NO: 53 - protein, 328 aa, synthetic construct
  source 1..328: note = CH
ASTKGPSVFPLAPSSKSTSGGTAALGCLVKDYFPEPVTVSWNSGALTSGVHTFPAVLQSSGLYSLSSVVTVPSSSLGTQTYICNVNHKPSNTKVDKRVEPKSCDKTHTCPPCPAPEAAGGPSVFLFPPKPKDTLMISRTPEVTCVVVDVEFEDPEVKFNWYVDGVEVHNAKTKPREEQYNSTYRVVSVLTVLHQDWLNGKEYKCKVTNKALPAPIEKTISKAKGQPREPQVYTLPPSREEMTKNQVSLTCLVKGFYPSDIAVEWESNGQPENNYKTTPPVLDSDGSFFLYSKLTVDKSRWQQGNVFSCSVMHEALHNHYTQKSLSLSP

SEQ ID NO: 54 - protein, 328 aa, synthetic construct
  source 1..328: note = CH
ASTKGPSVFPLAPSSKSTSGGTAALGCLVKDYFPEPVTVSWNSGALTSGVHTFPAVLQSSGLYSLSSVVTVPSSSLGTQTYICNVNHKPSNTKVDKRVEPKSCDKTHTCPPCPAPEAAGGPSVFLFPPKPKDTLMISRTPEVTCVVVDVSHEDPEVKFNWYVDGVEVHNAKTKPREEQYNSTYRVVSVLTVLHQDWLNGKEYKCKVSNAALPAPISKTISKAKGQPREPQVYTLPPSREEMTKNQVSLTCLVKGFYPSDIAVEWESNGQPENNYKTTPPVLDSDGSFFLYSKLTVDKSRWQQGNVFSCSVMHEALHNHYTQKSLSLSP

SEQ ID NO: 55 - protein, 328 aa, synthetic construct
  source 1..328: note = CH
ASTKGPSVFPLAPSSKSTSGGTAALGCLVKDYFPEPVTVSWNSGALTSGVHTFPAVLQSSGLYSLSSVVTVPSSSLGTQTYICNVNHKPSNTKVDKRVEPKSCDKTHTCPPCPAPEAAGGPSVFLFPPKPKDTLMISRTPEVTCVVVDVSHEDPEVKFNWYVDGVEVHNAKTKPREEQYNSTYRVVSVLTVLHQDWLNGKEYKCKVSNDALPAPISKTISKAKGQPREPQVYTLPPSREEMTKNQVSLTCLVKGFYPSDIAVEWESNGQPENNYKTTPPVLDSDGSFFLYSKLTVDKSRWQQGNVFSCSVMHEALHNHYTQKSLSLSP

SEQ ID NO: 56 - protein, 328 aa, synthetic construct
  source 1..328: note = CH
ASTKGPSVFPLAPSSKSTSGGTAALGCLVKDYFPEPVTVSWNSGALTSGVHTFPAVLQSSGLYSLSSVVTVPSSSLGTQTYICNVNHKPSNTKVDKRVEPKSCDKTHTCPPCPAPEAAGGPSVFLFPPKPKDTLMISRTPEVTCVVVDVSHEDPEVKFNWYVDGVEVHNAKTKPREEQYNSTYRVVSVLTVLHQDWLNGKEYKCKVSNEALPAPISKTISKAKGQPREPQVYTLPPSREEMTKNQVSLTCLVKGFYPSDIAVEWESNGQPENNYKTTPPVLDSDGSFFLYSKLTVDKSRWQQGNVFSCSVMHEALHNHYTQKSLSLSP

SEQ ID NO: 57 - protein, 328 aa, synthetic construct
  source 1..328: note = CH
ASTKGPSVFPLAPSSKSTSGGTAALGCLVKDYFPEPVTVSWNSGALTSGVHTFPAVLQSSGLYSLSSVVTVPSSSLGTQTYICNVNHKPSNTKVDKRVEPKSCDKTHTCPPCPAPEAAGGPSVFLFPPKPKDTLMISRTPEVTCVVVDVSHEDPEVKFNWYVDGVEVHNAKTKPREEQYNSTYRVVSVLTVLHQDWLNGKEYKCKVSNMALPAPISKTISKAKGQPREPQVYTLPPSREEMTKNQVSLTCLVKGFYPSDIAVEWESNGQPENNYKTTPPVLDSDGSFFLYSKLTVDKSRWQQGNVFSCSVMHEALHNHYTQKSLSLSP

SEQ ID NO: 58 - protein, 328 aa, synthetic construct
  source 1..328: note = CH
ASTKGPSVFPLAPSSKSTSGGTAALGCLVKDYFPEPVTVSWNSGALTSGVHTFPAVLQSSGLYSLSSVVTVPSSSLGTQTYICNVNHKPSNTKVDKRVEPKSCDKTHTCPPCPAPEAAGGPSVFLFPPKPKDTLMISRTPEVTCVVVDVSHEDPEVKFNWYVDGVEVHNAKTKPREEQYNSTYRVVSVLTVLHQDWLNGKEYKCKVSNAALPAPISKTISKAKGQPREPQVYTLPPSREEMTKNQVSLTCLVKGFYPSDIAVEWESNGQPENNYKTTPPVLDSDGSFFLYSKLTVDKSRWQQGNVFSCSVLHEALHAHTTRKELSLSP

SEQ ID NO: 59 - protein, 328 aa, synthetic construct
  source 1..328: note = CH
ASTKGPSVFPLAPSSKSTSGGTAALGCLVKDYFPEPVTVSWNSGALTSGVHTFPAVLQSSGLYSLSSVVTVPSSSLGTQTYICNVNHKPSNTKVDKRVEPKSCDKTHTCPPCPAPEAAGGPSVFLFPPKPKDTLMISRTPEVTCVVVDVSHEDPEVKFNWYVDGVEVHNAKTKPREEQYNSTYRVVSVLTVLHQDWLNGKEYKCKVSNAALPAPISKTISKAKGQPREPQVYTLPPSREEMTKNQVSLTCLVKGFYPSDIAVEWESNGQPENNYKTTPPVLDSDGSFFLYSKLTVDKSRWQQGNVFSCSVLHEALHAHYTRKELSLSP

SEQ ID NO: 60 - protein, 107 aa, synthetic construct [sequence omitted]

SEQ ID NO: 61 - protein, 585 aa, synthetic construct
  source 1..585: note = DENV
MKCLLYLAFLFIGVNCFHLTTRGGEPHMIVSKQERGKSLLFKTSAGVNMCTLIAMDLGELCEDTMTYKCPRITEAEPDDVDCWCNATDTWVTYGTCSQTGEHRRDKRSVALAPHVGLGLETRTETWMSSEGAWKQIQKVETWALRHPGFTVIALFLAHAIGTSITQKGIIFILLMLVTPSMAMRCVGIGNRDFVEGLSGATWVDVVLEHGSCVTTMAKNKPTLDIELLKTEVTNPAVLRKLCIEAKISNTTTDSRCPTQGEATLVEEQDANFVCRRTVVDRGWGNGCGLFGKGSLLTCAKFKCVTKLEGKIVQYENLKYSVIVTVHTGDQHQVGNETTEHGTIATITPQAPTSEIQLTDYGTLTLDCSPRTGLDFNEMVLLTMKEKSWLVHKQWFLDLPLPWTSGASTSQETWNRQDLLVTFKTAHAKKQEVVVLGSQEGAMHTALTGATEIQTSGTTTIFAGHLKCRLKMDKLTLKGMSYVMCTGSFKLEKEVAETQHGTVLVQVKYEGTDAPCKIPFSTQDEKGVTQNGRLITANPIVTDKEKPVNIETEPPFGESYIIVGAGEKALKLSWFKKGHHHHHHHH

SEQ ID NO: 62 - protein, 585 aa, synthetic construct
  source 1..585: note = DENV
MKCLLYLAFLFIGVNCFHLTTRNGEPHMIVSRQEKGKSLLFKTEDGVNMCTLMAMDLGELCEDTITYKCPFLRQNEPEDIDCWCNSTSTWVTYGTCTTTGEHRREKRSVALVPHVGMGLETRTETWMSSEGAWKHAQRIETWILRHPGFTIMAAILAYTIGTTHFQRALIFILLTAVAPSMTMRCIGISNRDFVEGVSGGSWVDIVLEHGSCVTTMAKNKPTLDFELIKTEAKQPATLRKYCIEAKLTNTTTDSRCPTQGEPSLNEEQDKRFVCKHSMVDRGWGNGCGLFGKGGIVTCAMFTCKKNMKGKVVQPENLEYTIVITPHSGEEHAVGNDTGKHGKEIKITPQSSITEAELTGYGTVTMECSPRTGLDFNEMVLLQMENKAWLVHRQWFLDLPLPWLPGADTQGSNWIQKETLVTFKNPHAKKQDVVVLGSQEGAMHTALTGATEIQMSSGNLLFTGHLKCRLRMDKLQLKGMSYSMCTGKFKVVKEIAETQHGTIVIRVQYEGDGSPCKIPFEIMDLEKRHVLGRLITVNPIVTEKDSPVNIEAEPPFGDSYIIIGVEPGQLKLNWFKKGHHHHHHHH

SEQ ID NO: 63 - protein, 583 aa, synthetic construct
  source 1..583: note = DENV
MKCLLYLAFLFIGVNCFHLTSRDGEPRMIVGKNERGKSLLFKTASGINMCTLIAMDLGEMCDDTVTYKCPHITEVEPEDIDCWCNLTSTWVTYGTCNQAGEHRRDKRSVALAPHVGMGLDTRTQTWMSAEGAWRQVEKVETWALRHPGFTILALFLAHYIGTSLTQKVVIFILLMLVTPSMTMRCVGVGNRDFVEGLSGATWVDVVLEHGGCVTTMAKNKPTLDIELQKTEATQLATLRKLCIEGKITNITTDSRCPTQGEAILPEEQDQNYVCKHTYVDRGWGNGCGLFGKGSLVTCAKFQCLESIEGKVVQHENLKYTVIITVHTGDQHQVGNETQGVTAEITSQASTAEAILPEYGTLGLECSPRTGLDFNEMILLTMKNKAWMVHRQWFFDLPLPWTSGATTKTPTWNRKELLVTFKNAHAKKQEVVVLGSQEGAMHTALTGATEIQTSGGTSIFAGHLKCRLKMDKLKLKGMSYAMCLNTFVLKKEVSETQHGTILIKVEYKGEDAPCKIPFSTEDGQGKAHNGRLITANPVVTKKEEPVNIEAEPPFGESNIVIGIGDKALKINWYRKGHHHHHHHH

SEQ ID NO: 64 - protein, 585 aa, synthetic construct
  source 1..585: note = DENV
MKCLLYLAFLFIGVNCFSLSTRDGEPLMIVAKHERGRPLLFKTTEGINKCTLIAMDLGEMCEDTVTYKCPLLVNTEPEDIDCWCNLTSTWVMYGTCTQSGERRREKRSVALTPHSGMGLETRAETWMSSEGAWKHAQRVESWILRNPGFALLAGFMAYMIGQTGIQRTVFFVLMMLVAPSYGMRCVGVGNRDFVEGVSGGAWVDLVLEHGGCVTTMAQGKPTLDFELTKTTAKEVALLRTYCIEASISNITTATRCPTQGEPYLKEEQDQQYICRRDVVDRGWGNGCGLFGKGGVVTCAKFSCSGKITGNLVQIENLEYTVVVTVHNGDTHAVGNDTSNHGVTAMITPRSPSVEVKLPDYGELTLDCEPRSGIDFNEMILMKMKKKTWLVHKQWFLDLPLPWTAGADTSEVHWNYKERMVTFKVPHAKRQDVTVLGSQEGAMHSALAGATEVDSGDGNHMFAGHLKCKVRMEKLRIKGMSYTMCSGKFSIDKEMAETQHGTTVVKVKYEGAGAPCKVPIEIRDVNKEKVVGRIISSTPLAENTNSVTNIELEPPFGDSYIVIGVGNSALTLHWFRKGHHHHHHHH

SEQ ID NO: 65 - protein, 403 aa, synthetic construct
  source 1..403: note = DENV
MRCVGIGNRDFVEGLSGATWVDVVLEHGSCVTTMAKNKPTLDIELLKTEVTNPAVLRKLCIEAKISNTTTDSRCPTQGEATLVEEQDANFVCRRTVVDRGWGNGCGLFGKGSLLTCAKFKCVTKLEGKIVQYENLKYSVIVTVHTGDQHQVGNETTEHGTIATITPQAPTSEIQLTDYGTLTLDCSPRTGLDFNEMVLLTMKEKSWLVHKQWFLDLPLPWTSGASTSQETWNRQDLLVTFKTAHAKKQEVVVLGSQEGAMHTALTGATEIQTSGTTTIFAGHLKCRLKMDKLTLKGMSYVMCTGSFKLEKEVAETQHGTVLVQVKYEGTDAPCKIPFSTQDEKGVTQNGRLITANPIVTDKEKPVNIETEPPFGESYIIVGAGEKALKLSWFKKGHHHHHHHH

SEQ ID NO: 66 - protein, 403 aa, synthetic construct
  source 1..403: note = DENV
MRCIGISNRDFVEGVSGGSWVDIVLEHGSCVTTMAKNKPTLDFELIKTEAKQPATLRKYCIEAKLTNTTTDSRCPTQGEPSLNEEQDKRFVCKHSMVDRGWGNGCGLFGKGGIVTCAMFTCKKNMKGKVVQPENLEYTIVITPHSGEEHAVGNDTGKHGKEIKITPQSSITEAELTGYGTVTMECSPRTGLDFNEMVLLQMENKAWLVHRQWFLDLPLPWLPGADTQGSNWIQKETLVTFKNPHAKKQDVVVLGSQEGAMHTALTGATEIQMSSGNLLFTGHLKCRLRMDKLQLKGMSYSMCTGKFKVVKEIAETQHGTIVIRVQYEGDGSPCKIPFEIMDLEKRHVLGRLITVNPIVTEKDSPVNIEAEPPFGDSYIIIGVEPGQLKLNWFKKGHHHHHHHH

SEQ ID NO: 67 - protein, 401 aa, synthetic construct
  source 1..401: note = DENV
MRCVGVGNRDFVEGLSGATWVDVVLEHGGCVTTMAKNKPTLDIELQKTEATQLATLRKLCIEGKITNITTDSRCPTQGEAILPEEQDQNYVCKHTYVDRGWGNGCGLFGKGSLVTCAKFQCLESIEGKVVQHENLKYTVIITVHTGDQHQVGNETQGVTAEITSQASTAEAILPEYGTLGLECSPRTGLDFNEMILLTMKNKAWMVHRQWFFDLPLPWTSGATTKTPTWNRKELLVTFKNAHAKKQEVVVLGSQEGAMHTALTGATEIQTSGGTSIFAGHLKCRLKMDKLKLKGMSYAMCLNTFVLKKEVSETQHGTILIKVEYKGEDAPCKIPFSTEDGQGKAHNGRLITANPVVTKKEEPVNIEAEPPFGESNIVIGIGDKALKINWYRKGHHHHHHHH

SEQ ID NO: 68 - protein, 403 aa, synthetic construct
  source 1..403: note = DENV
MRCVGVGNRDFVEGVSGGAWVDLVLEHGGCVTTMAQGKPTLDFELTKTTAKEVALLRTYCIEASISNITTATRCPTQGEPYLKEEQDQQYICRRDVVDRGWGNGCGLFGKGGVVTCAKFSCSGKITGNLVQIENLEYTVVVTVHNGDTHAVGNDTSNHGVTAMITPRSPSVEVKLPDYGELTLDCEPRSGIDFNEMILMKMKKKTWLVHKQWFLDLPLPWTAGADTSEVHWNYKERMVTFKVPHAKRQDVTVLGSQEGAMHSALAGATEVDSGDGNHMFAGHLKCKVRMEKLRIKGMSYTMCSGKFSIDKEMAETQHGTTVVKVKYEGAGAPCKVPIEIRDVNKEKVVGRIISSTPLAENTNSVTNIELEPPFGDSYIVIGVGNSALTLHWFRKGHHHHHHHH

SEQ ID NO: 69 - protein, 374 aa, Homo sapiens
MWFLTTLLLWVPVDGQVDTTKAVITLQPPWVSVFQEETVTLHCEVLHLPGSSSTQWFLNGTATQTSTPSYRITSASVNDSGEYRCQRGLSGRSDPIQLEIHRGWLLLQVSSRVFTEGEPLALRCHAWKDKLVYNVLYYRNGKAFKFFHWNSNLTILKTNISHNGTYHCSGMGKHRYTSAGISVTVKELFPAPVLNASVTSPLLEGNLVTLSCETKLLLQRPGLQLYFSFYMGSKTLRGRNTSSEYQILTARREDSGLYWCEAATEDGNVLKRSPELELQVLGLQLPTPVWFHVLFYLAVGIMFLVNTVLWVTIRKELKRKKKWDLEISLDSGHEKKVISSLQEDRHLEEELKCQEQKEEQLQEGVHRKEPQGAT

SEQ ID NO: 70 - protein, 316 aa, Homo sapiens
MTMETQMSQNVCPRNLWLLQPLTVLLLLASADSQAAPPKAVLKLEPPWINVLQEDSVTLTCQGARSPESDSIQWFHNGNLIPTHTQPSYRFKANNNDSGEYTCQTGQTSLSDPVHLTVLSEWLVLQTPHLEFQEGETIMLRCHSWKDKPLVKVTFFQNGKSQKFSHLDPTFSIPQANHSHSGDYHCTGNIGYTLFSSKPVTITVQVPSMGSSSPMGVIVAVVIATAVAAIVAAVVALIYCRKKRISANSTDPVKAAQFEPPGRQMIAIRKRQLEETNNDYETADGGYMTLNPRAPTDDDKNIYLTLPPNDHVNSNN

SEQ ID NO: 71 - protein, 316 aa, Homo sapiens
MTMETQMSQNVCPRNLWLLQPLTVLLLLASADSQAAPPKAVLKLEPPWINVLQEDSVTLTCQGARSPESDSIQWFHNGNLIPTHTQPSYRFKANNNDSGEYTCQTGQTSLSDPVHLTVLSEWLVLQTPHLEFQEGETIMLRCHSWKDKPLVKVTFFQNGKSQKFSRLDPTFSIPQANHSHSGDYHCTGNIGYTLFSSKPVTITVQVPSMGSSSPMGVIVAVVIATAVAAIVAAVVALIYCRKKRISANSTDPVKAAQFEPPGRQMIAIRKRQLEETNNDYETADGGYMTLNPRAPTDDDKNIYLTLPPNDHVNSNN

SEQ ID NO: 72 - protein, 291 aa, Homo sapiens
MGILSFLPVLATESDWADCKSPQPWGHMLLWTAVLFLAPVAGTPAAPPKAVLKLEPQWINVLQEDSVTLTCRGTHSPESDSIQWFHNGNLIPTHTQPSYRFKANNNDSGEYTCQTGQTSLSDPVHLTVLSEWLVLQTPHLEFQEGETIVLRCHSWKDKPLVKVTFFQNGKSKKFSRSDPNFSIPQANHSHSGDYHCTGNIGYTLYSSKPVTITVQAPSSSPMGIIVAVVTGIAVAAIVAAVVALIYCRKKRISANPTNPDEADKVGAENTITYSLLMHPDALEEPDDQNRI

SEQ ID NO: 73 - protein, 254 aa, Homo sapiens
MWQLLLPTALLLLVSAGMRTEDLPKAVVFLEPQWYRVLEKDSVTLKCQGAYSPEDNSTQWFHNESLISSQASSYFIDAATVDDSGEYRCQTNLSTLSDPVQLEVHIGWLLLQAPRWVFKEEDPIHLRCHSWKNTALHKVTYLQNGKGRKYFHHNSDFYIPKATLKDSGSYFCRGLFGSKNVSSETVNITITQGLSVSTISSFFPPGYQVSFCLVMVLLFAVDTGLYFSVKTNIRSSTRDWKDHKFKWRKDPQDK

SEQ ID NO: 74 - protein, 254 aa, Homo sapiens [sequence omitted]

SEQ ID NO: 75 - protein, 233 aa, Homo sapiens
MWQLLLPTALLLLVSAGMRTEDLPKAVVFLEPQWYRVLEKDSVTLKCQGAYSPEDNSTQWFHNENLISSQASSYFIDAATVDDSGEYRCQTNLSTLSDPVQLEVHVGWLLLQAPRWVFKEEDPIHLRCHSWKNTALHKVTYLQNGKDRKYFHHNSDFHIPKATLKDSGSYFCRGLVGSKNVSSETVNITITQGLAVSTISSFSPPGYQVSFCLVMVLLFAVDTGLYFSVKTNI

SEQ ID NO: 76 - protein, 233 aa, Homo sapiens
MWQLLLPTALLLLVSAGMRTEDLPKAVVFLEPQWYSVLEKDSVTLKCQGAYSPEDNSTQWFHNESLISSQASSYFIDAATVNDSGEYRCQTNLSTLSDPVQLEVHIGWLLLQAPRWVFKEEDPIHLRCHSWKNTALHKVTYLQNGKDRKYFHHNSDFHIPKATLKDSGSYFCRGLVGSKNVSSETVNITITQGLAVSTISSFSPPGYQVSFCLVMVLLFAVDTGLYFSVKTNI

SEQ ID NO: 77 - protein, 404 aa, Mus musculus
MILTSFGDDMWLLTTLLLWVPVGGEVVNATKAVITLQPPWVSIFQKENVTLWCEGPHLPGDSSTQWFINGTAVQISTPSYSIPEASFQDSGEYRCQIGSSMPSDPVQLQIHNDWLLLQASRRVLTEGEPLALRCHGWKNKLVYNVVFYRNGKSFQFSSDSEVAILKTNLSHSGIYHCSGTGRHRYTSAGVSITVKELFTTPVLRASVSSPFPEGSLVTLNCETNLLLQRPGLQLHFSFYVGSKILEYRNTSSEYHIARAEREDAGFYWCEVATEDSSVLKRSPELELQVLGPQSSAPVWFHILFYLSVGIMFSLNTVLYVKIHRLQREKKYNLEVPLVSEQGKKANSFQQVRSDGVYEEVTATASQTTPKEAPDGPRSSVGDCGPEQPEPLPPSDSTGAQTSQS

SEQ ID NO: 78 - protein, 293 aa, Mus musculus
MGILPFLLIPMESNWTVHVFSRTLCHMLLWTAVLNLAAGTHDLPKAVVKLEPPWIQVLKEDTVTLTCEGTHNPGNSSTQWFHNGRSIRSQVQASYTFKATVNDSGEYRCQMEQTRLSDPVDLGVISDWLLLQTPQLVFLEGETITLRCHSWRNKLLNRISFFHNEKSVRYHHYSSNFSIPKANHSHSGDYYCKGSLGRTLHQSKPVTITVQGPKSSRSLPVLTIVAAVTGIAVAAIVIILVSLVYLKKKQVPDNPPDLEEAAKTEAENTITYSLLKHPEALDEETEHDYQNHI

SEQ ID NO: 79 - protein, 267 aa, Mus musculus
MTLDTQMFQNAHSGSQWLLPPLTILLLFAFADRQSAALPKAVVKLDPPWIQVLKEDMVTLMCEGTHNPGNSSTQWFHNWSSIRSQVQSSYTFKATVNDSGEYRCQMEQTRLSDPVDLGVISDWLLLQTPQRVFLEGETITLRCHSWRNKLLNRISFFHNEKSVRYHHYKSNFSIPKANHSHSGDYYCKGSLGSTQHQSKPVTITVQDPATTSSISLVWYHTAFSLVMCLLFAVDTGLYFYVRRNLQTPRDYWRKSLSIRKHQAPQDK

SEQ ID NO: 80 - protein, 249 aa, Mus musculus
MWQLLLPTALVLTAFSGIQAGLQKAVVNLDPKWVRVLEEDSVTLRCQGTFSPEDNSIKWFHNESLIPHQDANYVIQSARVKDSGMYRCQTALSTISDPVQLEVHMGWLLLQTTKWLFQEGDPIHLRCHSWQNRPVRKVTYLQNGKGKKYFHENSELLIPKATHNDSGSYFCRGLIGHNNKSSASFRISLGDPGSPSMFPPWHQITFCLLIGLLFAIDTVLYFSVRRGLQSPVADYEEPKIQWSKEPQDK

SEQ ID NO: 81 - protein, 365 aa, Homo sapiens
MGVPRPQPWALGLLLFLLPGSLGAESHLSLLYHLTAVSSPAPGTPAFWVSGWLGPQQYLSYNSLRGEAEPCGAWVWENQVSWYWEKETTDLRIKEKLFLEAFKALGGKGPYTLQGLLGCELGPDNTSVPTAKFALNGEEFMNFDLKQGTWGGDWPEALAISQRWQQQDKAANKELTFLLFSCPHRLREHLERGRGNLEWKEPPSMRLKARPSSPGFSVLTCSAFSFYPPELQLRFLRNGLAAGTGQGDFGPNSDGSFHASSSLTVKSGDEHHYCCIVQHAGLAQPLRVELESPAKSSVLVVGIVIGVLLLTAAAVGGALLWRRMRSGLPAPWISLRGDDTGVLLPTPGEAQDADLKDVNVIPATA

SEQ ID NO: 82 - protein, 119 aa, Homo sapiens
MSRSVALAVLALLSLSGLEAIQRTPKIQVYSRHPAENGKSNFLNCYVSGFHPSDIEVDLLKNGERIEKVEHSDLSFSKDWSFYLLYYTEFTPTEKDEYACRVNHVTLSQPKIVKWDRDM

SEQ ID NO: 83 - protein, 330 aa, Homo sapiens [sequence omitted]

SEQ ID NO: 84 - protein, 326 aa, Homo sapiens
ASTKGPSVFPLAPCSRSTSESTAALGCLVKDYFPEPVTVSWNSGALTSGVHTFPAVLQSSGLYSLSSVVTVPSSNFGTQTYTCNVDHKPSNTKVDKTVERKCCVECPPCPAPPVAGPSVFLFPPKPKDTLMISRTPEVTCVVVDVSHEDPEVQFNWYVDGVEVHNAKTKPREEQFNSTFRVVSVLTVVHQDWLNGKEYKCKVSNKGLPAPIEKTISKTKGQPREPQVYTLPPSREEMTKNQVSLTCLVKGFYPSDIAVEWESNGQPENNYKTTPPMLDSDGSFFLYSKLTVDKSRWQQGNVFSCSVMHEALHNHYTQKSLSLSPGK

SEQ ID NO: 85 - protein, 377 aa, Homo sapiens
ASTKGPSVFPLAPCSRSTSGGTAALGCLVKDYFPEPVTVSWNSGALTSGVHTFPAVLQSSGLYSLSSVVTVPSSSLGTQTYTCNVNHKPSNTKVDKRVELKTPLGDTTHTCPRCPEPKSCDTPPPCPRCPEPKSCDTPPPCPRCPEPKSCDTPPPCPRCPAPELLGGPSVFLFPPKPKDTLMISRTPEVTCVVVDVSHEDPEVQFKWYVDGVEVHNAKTKPREEQYNSTFRVVSVLTVLHQDWLNGKEYKCKVSNKALPAPIEKTISKTKGQPREPQVYTLPPSREEMTKNQVSLTCLVKGFYPSDIAVEWESSGQPENNYNTTPPMLDSDGSFFLYSKLTVDKSRWQQGNIFSCSVMHEALHNRFTQKSLSLSPGK

SEQ ID NO: 86 - protein, 327 aa, Homo sapiens
ASTKGPSVFPLAPCSRSTSESTAALGCLVKDYFPEPVTVSWNSGALTSGVHTFPAVLQSSGLYSLSSVVTVPSSSLGTKTYTCNVDHKPSNTKVDKRVESKYGPPCPSCPAPEFLGGPSVFLFPPKPKDTLMISRTPEVTCVVVDVSQEDPEVQFNWYVDGVEVHNAKTKPREEQFNSTYRVVSVLTVLHQDWLNGKEYKCKVSNKGLPSSIEKTISKAKGQPREPQVYTLPPSQEEMTKNQVSLTCLVKGFYPSDIAVEWESNGQPENNYKTTPPVLDSDGSFFLYSRLTVDKSRWQEGNVFSCSVMHEALHNHYTQKSLSLSLGK

SEQ ID NO: 87 - protein, 328 aa, synthetic construct
  source 1..328: note = CH
ASTKGPSVFPLAPSSKSTSGGTAALGCLVKDYFPEPVTVSWNSGALTSGVHTFPAVLQSSGLYSLSSVVTVPSSSLGTQTYICNVNHKPSNTKVDKKVEPKSCDKTHTCPPCPAPELLGGPSVFLFPPKPKDTLMISRTPEVTCVVVDVSHEDPEVKFNWYVDGVEVHNAKTKPREEQYNSTYRVVSVLTVLHQDWLNGKEYKCKVSNKALPAPIEKTISKAKGQPREPQVYTLPPSREEMTKNQVSLTCLVKGFYPSDIAVEWESNGQPENNYKTTPPVLDSDGSFFLYSKLTVDKSRWQQGNVFSCSVMHEALHNHYTQKSLSLSP

SEQ ID NO: 88 - protein, 119 aa, synthetic construct
  source 1..119: note = VH
EVQLVESGGGSVKPGGSLKLSCAASGFTFSDHYMYWVRQTPEKRLEWVAIISGGGSYTSYPDSMKGRFTISRDNAKNILHLQMSSLKSEDTAMYYCTRESNGKPGFAYWGQGTLVTVSA

SEQ ID NO: 89 - protein, 111 aa, synthetic construct
  source 1..111: note = VL
DIELTQSPTSLAVSLGQRATISCKASQSVDYAGDSYMNWYQQKPGQPPKLLIYAASNLESGIPARFSASGSGTDFTLNIHPVEEEDAATYYCQQSYEDPWTFGGGTKLEIK

SEQ ID NO: 90 - protein, 132 aa, synthetic construct
  source 1..132: note = VH
QVQLVQSGPDVEKPGASVKVSCKASGYTFTSYYIHWVRQAPGQGLEWMGVINPRGGSRRSAQKFQGRITMTRDTSTSTVYMELSSLRSEDTAVYYCARGGRALFYDSYTTPFDGGSWWFDPWGQGSLVTVSS

SEQ ID NO: 91 - protein, 132 aa, synthetic construct
  source 1..132: note = VH
QVQLVQSGAEVKKPGASVKVSCKASGYTFTSNYIHWVRQAPGQGLEWMGVINPRGGSRRSAQKFQGRVTMTRDTSTSTVYMELSSLRSEDTAVYYCARGGRALFYDSYTTPFDGGSWWFDPWGQGSLVTVSS

SEQ ID NO: 92 - protein, 132 aa, synthetic construct
  source 1..132: note = VH
QVQLVQSGAEVKKPGASVKVSCKASGYTFTSYYIHWVRQAPGQGLEWMGVINPRGGSRRSAQKFQGRVTMTRDTSTSTVYMELSSLRSEDTAVYYCARGGRALFYDSYTTPFDGGSWWFDPWGQGSLVTVSS

SEQ ID NO: 93 - protein, 132 aa, synthetic construct
  source 1..132: note = VH
QVQLVQSGPDVEKPGASVKVSCKASGYTFTSYYMHWVRQAPGQGLEWMGVINPRGGSRRSAQKFQGRITMTRDTSTSTVYMELSSLRSEDTAVYYCARGGRALFYDSYTTPFDGGSWWFDPWGQGSLVTVSS

SEQ ID NO: 94 - protein, 132 aa, synthetic construct
  source 1..132: note = VH
QVQLVQSGAEVKKPGASVKVSCKASGYTFTSYYMHWVRQAPGQGLEWMGVINPRGGSRRSAQKFQGRVTMTRDTSTSTVYMELSSLRSEDTAVYYCARGGRALFYDSYTTPFDGGSWWFDPWGQGSLVTVSS

SEQ ID NO: 95 - protein, 132 aa, synthetic construct
  source 1..132: note = VH
QVQLVQSGAEVKKPGASVKVSCKASGYTFTSYYMHWVRQAPGQGLEWMGVINPRGGSRRSAQKFQGRVTMTRDTSTSTVYMELSSLRSEDTAVYYCARGGEALFYDSYTTPFDGGSWWFDPWGQGSLVTVSS

SEQ ID NO: 96 - protein, 107 aa, synthetic construct
  source 1..107: note = VL
DIQLTQSPSSLSASVGDRVTFTCQASQDIRKYLNWYQQKPGKAPKLLIYDASNLKTGVPSRFSGSGSGTDFTFTISSLQPEDVATYYCQQFEDLPITFGQGTRLQIK

SEQ ID NO: 97 - protein, 107 aa, synthetic construct
  source 1..107: note = VL
DIQLTQSPSSLSASVGDRVTFTCQASQEIRKYLNWYQQKPGKAPKLLIYDASNLKTGVPSRFSGSGSGTDFTFTISSLQPEDVATYYCQQFDDLPITFGQGTRLQIK

SEQ ID NO: 98 - protein, 107 aa, synthetic construct
  source 1..107: note = VL
DIQLTQSPSSLSASVGDRVTITCQASQDIRKYLNWYQQKPGKAPKLLIYDASNLKTGVPSRFSGSGSGTDFTLTISSLQPEDVATYYCQQFDDLPITFGQGTRLQIK

SEQ ID NO: 99 - protein, 107 aa, synthetic construct
  source 1..107: note = VL
DIQLTQSPSSLSASVGDRVTITCQASQEIRKYLNWYQQKPGKAPKLLIYDASNLKTGVPSRFSGSGSGTDFTLTISSLQPEDVATYYCQQFDDLPITFGQGTRLQIK

SEQ ID NO: 100 - protein, 107 aa, synthetic construct
  source 1..107: note = VL
DIQLTQSPSSLSASVGDRVTITCQASQDIRKYLNWYQQKPGKAPKLLIYDASNLKTGVPSRFSGSGSGTDFTLTISSLQPEDVATYYCQQFEDLPITFGQGTRLQIK

SEQ ID NO: 101 - protein, 5 aa, synthetic construct
  source 1..5: note = HVR-H1
SYYIH

SEQ ID NO: 102 - protein, 30 aa, synthetic construct
  source 1..30: note = FR-H1
QVQLVQSGAEVKKPGASVKVSCKASGYTFT

SEQ ID NO: 103 - protein, 32 aa, synthetic construct
  source 1..32: note = FR-H3
RVTMTRDTSTSTVYMELSSLRSEDTAVYYCAR

SEQ ID NO: 104 - protein, 23 aa, synthetic construct
  source 1..23: note = FR-L1
DIQLTQSPSSLSASVGDRVTITC

SEQ ID NO: 105 - protein, 32 aa, synthetic construct
  source 1..32: note = FR-L3
GVPSRFSGSGSGTDFTLTISSLQPEDVATYYC

SEQ ID NO: 106 - protein, 157 aa, synthetic construct
  source 1..157: note = CD154
DYKDDDDKMQKGDQNPQIAAHVISEASSKTTSVLQWAEKGYYTMSNNLVTLENGKQLTVKRQGLYYIYAQVTFCSNREASSQAPFIASLCLKSPGRFERILLRAANTHSSAKPCGQQSIHLGGVFELQPGASVFVNVTDPSQVSHGTGFTSFGLLKL

SEQ ID NO: 107 - protein, 328 aa, synthetic construct
  source 1..328: note = CH
ASTKGPSVFPLAPSSKSTSGGTAALGCLVKDYFPEPVTVSWNSGALTSGVHTFPAVLQSSGLYSLSSVVTVPSSSLGTQTYICNVNHKPSNTKVDKRVEPKSCDKTHTCPPCPAPELLGGPSVFLFPPKPKDTLMISRTPEVTCVVVDVSHEDPEVKFNWYVDGVEVHNAKTKPREEQYNSTYRVVSVLTVLHQDWLNGKEYKCKVSNAALPAPISKTISKAKGQPREPQVYTLPPSREEMTKNQVSLTCLVKGFYPSDIAVEWESNGQPENNYKTTPPVLDSDGSFFLYSKLTVDKSRWQQGNVFSCSVMHEALHNHYTQKSLSLSP

SEQ ID NO: 108 - protein, 328 aa, synthetic construct
  source 1..328: note = CH
ASTKGPSVFPLAPSSKSTSGGTAALGCLVKDYFPEPVTVSWNSGALTSGVHTFPAVLQSSGLYSLSSVVTVPSSSLGTQTYICNVNHKPSNTKVDKRVEPKSCDKTHTCPPCPAPEAAGGPSVFLFPPKPKDTLMISRTPEVTCVVVDVSHEDPEVKFNWYVDGVEVHNAKTKPREEQYNSTYRVVSVLTVLHQDWLNGKEYKCKVSNKALPAPIEKTISKAKGQPREPQVYTLPPSREEMTKNQVSLTCLVKGFYPSDIAVEWESNGQPENNYKTTPPVLDSDGSFFLYSKLTVDKSRWQQGNVFSCSVLHEALHAHTTRKELSLSP

SEQ ID NO: 109 - protein, 328 aa, synthetic construct
  source 1..328: note = CH
ASTKGPSVFPLAPSSKSTSGGTAALGCLVKDYFPEPVTVSWNSGALTSGVHTFPAVLQSSGLYSLSSVVTVPSSSLGTQTYICNVNHKPSNTKVDKRVEPKSCDKTHTCPPCPAPEAAGGPSVFLFPPKPKDTLMISRTPEVTCVVVDVSHEDPEVKFNWYVDGVEVHNAKTKPREEQYNSTYRVVSVLTVLHQDWLNGKEYKCKVSNKALPAPIEKTISKAKGQPREPQVYTLPPSREEMTKNQVSLTCLVKGFYPSDIAVEWESNGQPENNYKTTPPVLDSDGSFFLYSKLTVDKSRWQQGNVFSCSVLHEALHAHYTRKELSLSP